European Patent Specification EP 3 617 235 B1, published February 18, 2026. Title: Compounds and salts thereof comprising an affinity substance to a soluble protein, a clevable moiety, and a reactive group. Applicant: Ajinomoto Co., Inc. The sequence listing filed with the application follows.

SEQUENCE LISTING (105 sequences)

SEQ ID NO: 1 - protein, 230 aa, Artificial Sequence
  Fc region of human IgG1
  misc_feature (18)..(19): Xaa can be any naturally occurring amino acid
  misc_feature (21)..(21): Xaa can be any naturally occurring amino acid
  misc_feature (140)..(140): Xaa can be any naturally occurring amino acid
  misc_feature (142)..(142): Xaa can be any naturally occurring amino acid
  misc_feature (177)..(177): Xaa can be any naturally occurring amino acid
PKSCDKTHTCPPCPAPEXXGXPSVFLFPPKPKDTLMISRTPEVTCVVVDVSHEDPEVKFNWYVDGVEVHNAKTKPREEQYDSTYRVVSVLTVLHQDWLNGKEYKCKVSNKALPAPIEKTISKAKGQPREPQVYTLPPSRXEXTKNQVSLTCLVKGFYPSDIAVEWESNGQPENNYKXTPPVLDSDGSFFLYSKLTVDKSRWQQGNVFSCSVMHEALHNHYTQKSLSLSPG

SEQ ID NO: 2 - protein, 449 aa, Artificial Sequence
  Heavy chain of Trastuzumab (humanized IgG1 monoclonal antibody)
EVQLVESGGGLVQPGGSLRLSCAASGFNIKDTYIHWVRQAPGKGLEWVARIYPTNGYTRYADSVKGRFTISADTSKNTAYLQMNSLRAEDTAVYYCSRWGGDGFYAMDYWGQGTLVTVSSASTKGPSVFPLAPSSKSTSGGTAALGCLVKDYFPEPVTVSWNSGALTSGVHTFPAVLQSSGLYSLSSVVTVPSSSLGTQTYICNVNHKPSNTKVDKKVEPKSCDKTHTCPPCPAPELLGGPSVFLFPPKPKDTLMISRTPEVTCVVVDVSHEDPEVKFNWYVDGVEVHNAKTKPREEQYDSTYRVVSVLTVLHQDWLNGKEYKCKVSNKALPAPIEKTISKAKGQPREPQVYTLPPSREEMTKNQVSLTCLVKGFYPSDIAVEWESNGQPENNYKTTPPVLDSDGSFFLYSKLTVDKSRWQQGNVFSCSVMHEALHNHYTQKSLSLSPG

SEQ ID NO: 3 - protein, 237 aa, Artificial Sequence
  Fc region of human IgG1 antibody
IEGRMDPKSCDKTHTCPPCPAPEAEGAPSVFLFPPKPKDTLMISRTPEVTCVVVDVSHEDPEVKFNWYVDGVEVHNAKTKPREEQYDSTYRVVSVLTVLHQDWLNGKEYKCKVSNKALPAPIEKTISKAKGQPREPQVYTLPPSRDELTKNQVSLTCLVKGFYPSDIAVEWESNGQPENNYKATPPVLDSDGSFFLYSKLTVDKSRWQQGNVFSCSVMHEALHNHYTQKSLSLSPGK

SEQ ID NO: 4 - protein, 214 aa, Artificial Sequence
  Light chain of Trastuzumab (humanized IgG1 monoclonal antibody)
DIQMTQSPSSLSASVGDRVTITCRASQDVNTAVAWYQQKPGKAPKLLIYSASFLYSGVPSRFSGSRSGTDFTLTISSLQPEDFATYYCQQHYTTPPTFGQGTKVEIKRTVAAPSVFIFPPSDEQLKSGTASVVCLLNNFYPREAKVQWKVDNALQSGNSQESVTEQDSKDSTYSLSSTLTLSKADYEKHKVYACEVTHQGLSSPVTKSFNRGEC

SEQ ID NO: 5 - protein, 26 aa, Artificial Sequence
  Peptide fragment of Trastuzumab
THTCPPCPAPELLGGPSVFLFPPKPK

SEQ ID NO: 6 - protein, 16 aa, Artificial Sequence
  Peptide fragment of Trastuzumab
LLGGPSVFLFPPKPKD

SEQ ID NO: 7 - protein, 26 aa, Artificial Sequence
  Peptide fragment of Fc region of human IgG1 antibody
THTCPPCPAPEAEGAPSVFLFPPKPK

SEQ ID NO: 8 - protein, 24 aa, Artificial Sequence
  Peptide fragment of Fc region of human IgG1 antibody
GAPSVFLFPPKPKKDTLMISRTPE

SEQ ID NO: 9 - protein, 12 aa, Artificial Sequence
  Peptide having an affinity to CH2 region of human IgG
EPIHRSTLTALL

SEQ ID NO: 10 - protein, 10 aa, Artificial Sequence
  Peptide having an affinity to Fc region of human IgG
FARLVSSIRY

SEQ ID NO: 11 - protein, 10 aa, Artificial Sequence
  Peptide having an affinity to Fc region of human IgG
FGRLVSSIRY

SEQ ID NO: 12 - protein, 10 aa, Artificial Sequence
  Peptide having an affinity to Fc region of human IgG
TWKTSRISIF

SEQ ID NO: 13 - protein, 4 aa, Artificial Sequence
  Peptide having an affinity to specific region of human IgG
QSYP

SEQ ID NO: 14 - protein, 6 aa, Artificial Sequence
  Peptide having an affinity to Fc region of human IgG
HWRGWV

SEQ ID NO: 15 - protein, 6 aa, Artificial Sequence
  Peptide having an affinity to Fc region of human IgG
HYFKFD

SEQ ID NO: 16 - protein, 6 aa, Artificial Sequence
  Peptide having an affinity to Fc region of human IgG
HFRRHL

SEQ ID NO: 17 - protein, 4 aa, Artificial Sequence
  Peptide having an affinity to Fc region of human IgG
DAAG

SEQ ID NO: 18 - protein, 8 aa, Artificial Sequence
  Peptide having an affinity to Fc region of human IgG
NARKFYKG

SEQ ID NO: 19 - protein, 8 aa, Artificial Sequence
  Peptide having an affinity to Fc region of human IgG
NKFRGKYK

SEQ ID NO: 20 - protein, 13 aa, Artificial
  IgG-binding peptide
  misc_feature (6)..(6): Xaa is lysine, aspartic acid, glutamic acid, 2-amino suberic acid, or diaminopropionic acid
DCAYHXGELVWCT

SEQ ID NO: 21 - protein, 17 aa, Artificial
  IgG-binding peptide
  misc_feature (8)..(8): Xaa is lysine, aspartic acid, glutamic acid, 2-amino suberic acid, or diaminopropionic acid
GPDCAYHXGELVWCTFH

SEQ ID NO: 22 - protein, 13 aa, Artificial
  IgG-binding peptide
  misc_feature (6)..(6): Xaa is lysine, aspartic acid, glutamic acid, 2-amino suberic acid, or diaminopropionic acid
RCAYHXGELVWCS

SEQ ID NO: 23 - protein, 17 aa, Artificial
  IgG-binding peptide
  misc_feature (8)..(8): Xaa is lysine, aspartic acid, glutamic acid, 2-amino suberic acid, or diaminopropionic acid
GPRCAYHXGELVWCSFH

SEQ ID NO: 24 - protein, 17 aa, Artificial
  IgG-binding peptide
  misc_feature (8)..(8): Xaa is lysine, aspartic acid, glutamic acid, 2-amino suberic acid, or diaminopropionic acid
SPDCAYHXGELVWCTFH

SEQ ID NO: 25 - protein, 17 aa, Artificial
  IgG-binding peptide
  misc_feature (8)..(8): Xaa is lysine, aspartic acid, glutamic acid, 2-amino suberic acid, or diaminopropionic acid
GDDCAYHXGELVWCTFH

SEQ ID NO: 26 - protein, 17 aa, Artificial
  IgG-binding peptide
  misc_feature (8)..(8): Xaa is lysine, aspartic acid, glutamic acid, 2-amino suberic acid, or diaminopropionic acid
GPSCAYHXGELVWCTFH

SEQ ID NO: 27 - protein, 17 aa, Artificial
  IgG-binding peptide
  misc_feature (8)..(8): Xaa is lysine, aspartic acid, glutamic acid, 2-amino suberic acid, or diaminopropionic acid
GPDCAYHXGELVWCSFH

SEQ ID NO: 28 - protein, 17 aa, Artificial
  IgG-binding peptide
  misc_feature (8)..(8): Xaa is lysine, aspartic acid, glutamic acid, 2-amino suberic acid, or diaminopropionic acid
GPDCAYHXGELVWCTHH

SEQ ID NO: 29 - protein, 17 aa, Artificial
  IgG-binding peptide
  misc_feature (8)..(8): Xaa is lysine, aspartic acid, glutamic acid, 2-amino suberic acid, or diaminopropionic acid
GPDCAYHXGELVWCTFY

SEQ ID NO: 30 - protein, 17 aa, Artificial
  IgG-binding peptide
  misc_feature (8)..(8): Xaa is lysine, aspartic acid, glutamic acid, 2-amino suberic acid, or diaminopropionic acid
SPDCAYHXGELVWCTFY

SEQ ID NO: 31 - protein, 17 aa, Artificial
  IgG-binding peptide
  misc_feature (8)..(8): Xaa is lysine, aspartic acid, glutamic acid, 2-amino suberic acid, or diaminopropionic acid
SDDCAYHXGELVWCTFY

SEQ ID NO: 32 - protein, 17 aa, Artificial
  IgG-binding peptide
  misc_feature (8)..(8): Xaa is lysine, aspartic acid, glutamic acid, 2-amino suberic acid, or diaminopropionic acid
RGNCAYHXGQLVWCTYH

SEQ ID NO: 33 - protein, 17 aa, Artificial
  IgG-binding peptide
  misc_feature (2)..(2): Xaa is homoserine
  misc_feature (8)..(8): Xaa is lysine, aspartic acid, glutamic acid, 2-amino suberic acid, or diaminopropionic acid
  misc_feature (16)..(16): Xaa is homoserine
GXDCAYHXGELVWCTXH

SEQ ID NO: 34 - protein, 19 aa, Artificial
  IgG-binding peptide
  misc_feature (10)..(10): Xaa is lysine, aspartic acid, glutamic acid, 2-amino suberic acid, or diaminopropionic acid
RRGPDCAYHXGELVWCTFH

SEQ ID NO: 35 - protein, 13 aa, Artificial
  IgG-binding peptide
  misc_feature (6)..(6): Xaa is lysine, aspartic acid, glutamic acid, 2-amino suberic acid, or diaminopropionic acid
DCTYHXGNLVWCT

SEQ ID NO: 36 - protein, 13 aa, Artificial
  IgG-binding peptide
  misc_feature (6)..(6): Xaa is lysine, aspartic acid, glutamic acid, 2-amino suberic acid, or diaminopropionic acid
DCAYHXGNLVWCT

SEQ ID NO: 37 - protein, 13 aa, Artificial
  IgG-binding peptide
  misc_feature (6)..(6): Xaa is lysine, aspartic acid, glutamic acid, 2-amino suberic acid, or diaminopropionic acid
DCTYHXGELVWCT

SEQ ID NO: 38 - protein, 13 aa, Artificial
  IgG-binding peptide
  misc_feature (6)..(6): Xaa is lysine, aspartic acid, glutamic acid, 2-amino suberic acid, or diaminopropionic acid
DCAWHXGELVWCT

SEQ ID NO: 39 - protein, 17 aa, Artificial Sequence
  Arginine residue at N-terminus may be acetylated and two cysteine residues may be linked by disulfide bridge
RGNCAYHKGQLVWCTYH

SEQ ID NO: 40 - protein, 33 aa, Artificial Sequence
  peptide fragment of Trastuzumab (humanized IgG1 monoclonal antibody)
THTCPPCPAPELLGGPSVFLFPPKPKDTLMISR

SEQ ID NO: 41 - protein, 449 aa, Artificial Sequence
  Heavy chain of Trastuzumab (humanized IgG1 monoclonal antibody)
EVQLVESGGGLVQPGGSLRLSCAASGFNIKDTYIHWVRQAPGKGLEWVARIYPTNGYTRYADSVKGRFTISADTSKNTAYLQMNSLRAEDTAVYYCSRWGGDGFYAMDYWGQGTLVTVSSASTKGPSVFPLAPSSKSTSGGTAALGCLVKDYFPEPVTVSWNSGALTSGVHTFPAVLQSSGLYSLSSVVTVPSSSLGTQTYICNVNHKPSNTKVDKKVEPKSCDKTHTCPPCPAPELLGGPSVFLFPPKPKDTLMISRTPEVTCVVVDVSHEDPEVKFNWYVDGVEVHNAKTKPREEQYNSTYRVVSVLTVLHQDWLNGKEYKCKVSNKALPAPIEKTISKAKGQPREPQVYTLPPSREEMTKNQVSLTCLVKGFYPSDIAVEWESNGQPENNYKTTPPVLDSDGSFFLYSKLTVDKSRWQQGNVFSCSVMHEALHNHYTQKSLSLSPG

SEQ ID NO: 42 - protein, 17 aa, Artificial Sequence
  Arginine residue at N-terminus may be acetylated and two cysteine residues may be linked by disulfide bridge
RGNCKYHRGQLVWCTYH

SEQ ID NO: 43 - protein, 17 aa, Artificial Sequence
  Arginine residue at N-terminus may be acetylated and two cysteine residues may be linked by disulfide bridge
RGNCAWHRGKLVWCTYH

SEQ ID NO: 44 - protein, 17 aa, Artificial Sequence
  Arginine residue at N-terminus may be acetylated and two cysteine residues may be linked by disulfide bridge
RGNCKWHRGELVWCTYH

SEQ ID NO: 45 - protein, 17 aa, Artificial Sequence
  Arginine residue at N-terminus may be acetylated and two cysteine residues may be linked by disulfide bridge
RGNCKWHRGQLVWCTYH

SEQ ID NO: 46 - protein, 17 aa, Artificial Sequence
  Arginine residue at N-terminus may be acetylated and two cysteine residues may be linked by disulfide bridge
RGNCKYHLGELVWCTYH

SEQ ID NO: 47 - protein, 17 aa, Artificial Sequence
  Arginine residue at N-terminus may be acetylated and two cysteine residues may be linked by disulfide bridge
RGNCKYHLGQLVWCTYH

SEQ ID NO: 48 - protein, 13 aa, Artificial Sequence
  Aspartic acid residue at N-terminus may be acetylated and two cysteine residues may be linked by disulfide bridge
DCKWHLGELVWCT

SEQ ID NO: 49 - protein, 13 aa, Artificial Sequence
  Aspartic acid residue at N-terminus may be acetylated and two cysteine residues may be linked by disulfide bridge
DCKYHLGELVWCT

SEQ ID NO: 50 - protein, 13 aa, Artificial Sequence
  Aspartic acid residue at N-terminus may be acetylated and two cysteine residues may be linked by disulfide bridge
DCKWHRGELVWCT

SEQ ID NO: 51 - protein, 13 aa, Artificial Sequence
  Aspartic acid residue at N-terminus may be acetylated and two cysteine residues may be linked by disulfide bridge
DCKWHLGQLVWCT

SEQ ID NO: 52 - protein, 13 aa, Artificial Sequence
  Aspartic acid residue at N-terminus may be acetylated and two cysteine residues may be linked by disulfide bridge
DCKYHRGELVWCT

SEQ ID NO: 53 - protein, 13 aa, Artificial Sequence
  Aspartic acid residue at N-terminus may be acetylated and two cysteine residues may be linked by disulfide bridge
DCKYHLGQLVWCT

SEQ ID NO: 54 - protein, 13 aa, Artificial Sequence
  Aspartic acid residue at N-terminus may be acetylated and two cysteine residues may be linked by disulfide bridge
DCKWHRGQLVWCT

SEQ ID NO: 55 - protein, 13 aa, Artificial Sequence
  Aspartic acid residue at N-terminus may be acetylated and two cysteine residues may be linked by disulfide bridge
DCKYHRGQLVWCT

SEQ ID NO: 56 - protein, 17 aa, Artificial Sequence
  Arginine residue at N-terminus may be acetylated and two cysteine residues may be linked by disulfide bridge
RGNCAWHLGQLVWCKYH

SEQ ID NO: 57 - protein, 17 aa, Artificial Sequence
  Arginine residue at N-terminus may be acetylated and two cysteine residues may be linked by disulfide bridge
RGNCAWHLGELVWCKYH

SEQ ID NO: 58 - protein, 17 aa, Artificial Sequence
  Arginine residue at N-terminus may be acetylated and two cysteine residues may be linked by disulfide bridge
RGNCAYHLGQLVWCTKH

SEQ ID NO: 59 - protein, 17 aa, Artificial Sequence
  Arginine residue at N-terminus may be acetylated and two cysteine residues may be linked by disulfide bridge
RGNCAYHLGQLVWCTYK

SEQ ID NO: 60 - protein, 17 aa, Artificial Sequence
  Arginine residue at N-terminus may be acetylated and two cysteine residues may be linked by disulfide bridge
RGNCAYHRGQLVWCTKH

SEQ ID NO: 61 - protein, 34 aa, Artificial Sequence
  Lysine residue at N-terminus may be acetylated and two cysteine residues may be linked by disulfide bridge
KNMQCQRRFYEALHDPNLNEEQRNARIRSIRDDC

SEQ ID NO: 62 - protein, 34 aa, Artificial Sequence
  Phenylalanine residue at N-terminus may be acetylated and two cysteine residues may be linked by disulfide bridge
FNMQCQKRFYEALHDPNLNEEQRNARIRSIRDDC

SEQ ID NO: 63 - protein, 34 aa, Artificial Sequence
  Phenylalanine residue at N-terminus may be acetylated and two cysteine residues may be linked by disulfide bridge
FNMQCQRRFYEAKHDPNLNEEQRNARIRSIRDDC

SEQ ID NO: 64 - protein, 34 aa, Artificial Sequence
  Phenylalanine residue at N-terminus may be acetylated and two cysteine residues may be linked by disulfide bridge
FNMQCQRRFYEALHDPNLNEEQRKARIRSIRDDC

SEQ ID NO: 65 - protein, 34 aa, Artificial Sequence
  Phenylalanine residue at N-terminus may be acetylated and two cysteine residues may be linked by disulfide bridge
FNMQCQRRFYEALHDPNLNKEQRNARIRSIRDDC

SEQ ID NO: 66 - protein, 19 aa, Artificial Sequence
  Polypeptide fragment
VVSVLTVLHQDWLNGKEYK

SEQ ID NO: 67 - protein, 28 aa, Artificial Sequence
  Polypeptide fragment
EEQYDSTYRVVSVLTVLHQDWLNGKEYK

SEQ ID NO: 68 - protein, 34 aa, Artificial Sequence
  Phenylalanine residue at N-terminus may be acetylated and two cysteine residues may be linked by disulfide bridge
FNMQCQRRFYEALHDPNLNEEQRNARIRSIKDDC

SEQ ID NO: 69 - protein, 18 aa, Artificial Sequence
  Polypeptide fragment
FNWYVDGVEVHNAKTKPR

SEQ ID NO: 70 - protein, 34 aa, Artificial Sequence
  Phenylalanine residue at N-terminus may be acetylated and two cysteine residues may be linked by disulfide bridge
FNKQCQRRFYEALHDPNLNEEQRNARIRSIRDDC

SEQ ID NO: 71 - protein, 34 aa, Artificial Sequence
  Phenylalanine residue at N-terminus may be acetylated and two cysteine residues may be linked by disulfide bridge
FNMQCKRRFYEALHDPNLNEEQRNARIRSIRDDC

SEQ ID NO: 72 - protein, 34 aa, Artificial Sequence
  Phenylalanine residue at N-terminus may be acetylated and two cysteine residues may be linked by disulfide bridge
FNMQCQRRFYEALHDPNLNEEQRNARIRSIRKDC

SEQ ID NO: 73 - protein, 17 aa, Artificial Sequence
  Peptide having an affinity to Fc region of human IgG
  MISC_FEATURE (8)..(8): Xaa is arginine, leucine, lysine, aspartic acid, glutamic acid, 2-amino suberic acid, or diaminopropionic acid
RGNCAYHXGQLVWCTYH

SEQ ID NO: 74 - protein, 17 aa, Artificial Sequence
  Peptide having an affinity to Fc region of human IgG
  MISC_FEATURE (8)..(8): Xaa is arginine, leucine, lysine, aspartic acid, glutamic acid, 2-amino suberic acid, or diaminopropionic acid
RGNCAWHXGQLVWCTYH

SEQ ID NO: 75 - protein, 17 aa, Artificial Sequence
  Peptide having an affinity to Fc region of human IgG
  MISC_FEATURE (8)..(8): Xaa is arginine, leucine, lysine, aspartic acid, glutamic acid, 2-amino suberic acid, or diaminopropionic acid
RGNCAWHXGELVWCTYH

SEQ ID NO: 76 - protein, 17 aa, Artificial Sequence
  Peptide having an affinity to Fc region of human IgG
  MISC_FEATURE (8)..(8): Xaa is arginine, leucine, lysine, aspartic acid, glutamic acid, 2-amino suberic acid, or diaminopropionic acid
RGNCKWHXGQLVWCTYH

SEQ ID NO: 77 - protein, 17 aa, Artificial Sequence
  Peptide having an affinity to Fc region of human IgG
  MISC_FEATURE (8)..(8): Xaa is arginine, leucine, lysine, aspartic acid, glutamic acid, 2-amino suberic acid, or diaminopropionic acid
RGNCKYHXGELVWCTYH

SEQ ID NO: 78 - protein, 17 aa, Artificial Sequence
  Peptide having an affinity to Fc region of human IgG
  MISC_FEATURE (8)..(8): Xaa is arginine, leucine, lysine, aspartic acid, glutamic acid, 2-amino suberic acid, or diaminopropionic acid
RGNCKYHXGQLVWCTYH

SEQ ID NO: 79 - protein, 13 aa, Artificial Sequence
  Peptide having an affinity to Fc region of human IgG
  MISC_FEATURE (6)..(6): Xaa is arginine, leucine, lysine, aspartic acid, glutamic acid, 2-amino suberic acid, or diaminopropionic acid
DCKWHXGELVWCT

SEQ ID NO: 80 - protein, 13 aa, Artificial Sequence
  Peptide having an affinity to Fc region of human IgG
  MISC_FEATURE (6)..(6): Xaa is arginine, leucine, lysine, aspartic acid, glutamic acid, 2-amino suberic acid, or diaminopropionic acid
DCKYHXGELVWCT

SEQ ID NO: 81 - protein, 13 aa, Artificial Sequence
  Peptide having an affinity to Fc region of human IgG
  misc_feature (6)..(6): Xaa can be any naturally occurring amino acid
  MISC_FEATURE (8)..(8): Xaa is arginine, leucine, lysine, aspartic acid, glutamic acid, 2-amino suberic acid, or diaminopropionic acid
DCKWHXGELVWCT

SEQ ID NO: 82 - protein, 13 aa, Artificial Sequence
  Peptide having an affinity to Fc region of human IgG
  MISC_FEATURE (6)..(6): Xaa is arginine, leucine, lysine, aspartic acid, glutamic acid, 2-amino suberic acid, or diaminopropionic acid
DCKWHXGQLVWCT

SEQ ID NO: 83 - protein, 13 aa, Artificial Sequence
  Peptide having an affinity to Fc region of human IgG
  MISC_FEATURE (6)..(6): Xaa is arginine, leucine, lysine, aspartic acid, glutamic acid, 2-amino suberic acid, or diaminopropionic acid
DCKYHXGELVWCT

SEQ ID NO: 84 - protein, 13 aa, Artificial Sequence
  Peptide having an affinity to Fc region of human IgG
  MISC_FEATURE (6)..(6): Xaa is arginine, leucine, lysine, aspartic acid, glutamic acid, 2-amino suberic acid, or diaminopropionic acid
DCKYHXGQLVWCT

SEQ ID NO: 85 - protein, 13 aa, Artificial Sequence
  Peptide having an affinity to Fc region of human IgG
  MISC_FEATURE (6)..(6): Xaa is arginine, leucine, lysine, aspartic acid, glutamic acid, 2-amino suberic acid, or diaminopropionic acid
DCKWHXGQLVWCT

SEQ ID NO: 86 - protein, 13 aa, Artificial Sequence
  Peptide having an affinity to Fc region of human IgG
  MISC_FEATURE (6)..(6): Xaa is arginine, leucine, lysine, aspartic acid, glutamic acid, 2-amino suberic acid, or diaminopropionic acid
DCKYHXGQLVWCT

SEQ ID NO: 87 - protein, 17 aa, Artificial Sequence
  Peptide having an affinity to Fc region of human IgG
  MISC_FEATURE (8)..(8): Xaa is arginine, leucine, lysine, aspartic acid, glutamic acid, 2-amino suberic acid, or diaminopropionic acid
RGNCAWHXGQLVWCKYH

SEQ ID NO: 88 - protein, 17 aa, Artificial Sequence
  Peptide having an affinity to Fc region of human IgG
  MISC_FEATURE (8)..(8): Xaa is arginine, leucine, lysine, aspartic acid, glutamic acid, 2-amino suberic acid, or diaminopropionic acid
RGNCAWHXGELVWCKYH

SEQ ID NO: 89 - protein, 17 aa, Artificial Sequence
  Peptide having an affinity to Fc region of human IgG
  MISC_FEATURE (8)..(8): Xaa is arginine, leucine, lysine, aspartic acid, glutamic acid, 2-amino suberic acid, or diaminopropionic acid
RGNCAYHXGQLVWCTKH

SEQ ID NO: 90 - protein, 17 aa, Artificial Sequence
  Peptide having an affinity to Fc region of human IgG
  MISC_FEATURE (8)..(8): Xaa is arginine, leucine, lysine, aspartic acid, glutamic acid, 2-amino suberic acid, or diaminopropionic acid
RGNCAYHXGQLVWCTYK

SEQ ID NO: 91 - protein, 17 aa, Artificial Sequence
  Peptide having an affinity to Fc region of human IgG
  MISC_FEATURE (8)..(8): Xaa is arginine, leucine, lysine, aspartic acid, glutamic acid, 2-amino suberic acid, or diaminopropionic acid
RGNCAYHXGQLVWCTKH

SEQ ID NO: 92 - protein, 34 aa, Artificial Sequence
  Phenylalanine residue at N-terminus may be acetylated and two cysteine residues may be linked by disulfide bridge
FNMQCQRRFYEALHDPNLNEEQRNARIRSIRDDC

SEQ ID NO: 93 - protein, 34 aa, Artificial Sequence
  Phenylalanine residue at N-terminus may be acetylated and two cysteine residues may be linked by disulfide bridge
FNMQCQRRFYEALHDPNLNEEQRNAKIKSIRDDC

SEQ ID NO: 94 - protein, 17 aa, Artificial Sequence
  Peptide having an affinity to Fc region of human IgG
  misc_feature (1)..(3): Xaa can be any naturally occurring amino acid
  misc_feature (5)..(6): Xaa can be any naturally occurring amino acid
  MISC_FEATURE (8)..(8): Xaa is arginine, leucine, lysine, aspartic acid, glutamic acid, 2-amino suberic acid, or diaminopropionic acid
  MISC_FEATURE (10)..(10): Xaa is lysine, glutamine, glutamic acid, asparagine, or aspartic acid
  misc_feature (15)..(17): Xaa can be any naturally occurring amino acid
XXXCXXHXGXLVWCXXX

SEQ ID NO: 95 - protein, 17 aa, Artificial Sequence
  Peptide having an affinity to Fc region of human IgG
  misc_feature (1)..(3): Xaa can be any naturally occurring amino acid
  misc_feature (5)..(6): Xaa can be any naturally occurring amino acid
  MISC_FEATURE (8)..(8): Xaa is lysine, cystein, aspartic acid, glutamic acid, 2-amino suberic acid, or diaminopropionic acid
  MISC_FEATURE (10)..(10): Xaa is glutamic acid, or aspartic acid
  misc_feature (15)..(17): Xaa can be any naturally occurring amino acid
XXXCXXHXGXLVWCXXX

SEQ ID NO: 96 - protein, 17 aa, Artificial Sequence
  Peptide having an affinity to Fc region of human IgG
  misc_feature (1)..(3): Xaa can be any naturally occurring amino acid
  misc_feature (5)..(6): Xaa can be any naturally occurring amino acid
  MISC_FEATURE (8)..(8): Xaa is arginine, or leucine
  MISC_FEATURE (10)..(10): Xaa is lysine, glutamic acid, or aspartic acid
  misc_feature (15)..(17): Xaa can be any naturally occurring amino acid
XXXCXXHXGXLVWCXXX

SEQ ID NO: 97 - protein, 17 aa, Artificial Sequence
  Peptide having an affinity to Fc region of human IgG
  misc_feature (1)..(3): Xaa can be any naturally occurring amino acid
  misc_feature (5)..(5): Xaa can be any naturally occurring amino acid
  MISC_FEATURE (8)..(8): Xaa is lysine, cystein, aspartic acid, glutamic acid, 2-amino suberic acid, or diaminopropionic acid
  misc_feature (15)..(17): Xaa can be any naturally occurring amino acid
XXXCXYHXGNLVWCXXX

SEQ ID NO: 98 - protein, 17 aa, Artificial Sequence
  Peptide having an affinity to Fc region of human IgG
  misc_feature (1)..(3): Xaa can be any naturally occurring amino acid
  misc_feature (6)..(6): Xaa can be any naturally occurring amino acid
  MISC_FEATURE (8)..(8): Xaa is arginine, leucine, lysine, cystein, aspartic acid, glutamic acid, 2-amino suberic acid, or diaminopropionic acid
  misc_feature (15)..(17): Xaa can be any naturally occurring amino acid
XXXCAXHXGELVWCXXX

SEQ ID NO: 99 - protein, 17 aa, Artificial Sequence
  Peptide having an affinity to Fc region of human IgG
  misc_feature (1)..(3): Xaa can be any naturally occurring amino acid
  MISC_FEATURE (5)..(5): Xaa is alanine, serine, or threonine
  MISC_FEATURE (6)..(6): Xaa is tyrosine, or tryptophan
  MISC_FEATURE (8)..(8): Xaa is lysine, cystein, aspartic acid, glutamic acid, 2-amino suberic acid, or diaminopropionic acid
  MISC_FEATURE (10)..(10): Xaa is glutamic acid, or aspartic acid
  misc_feature (15)..(17): Xaa can be any naturally occurring amino acid
XXXCXXHXGXLVWCXXX

SEQ ID NO: 100 - protein, 17 aa, Artificial Sequence
  Peptide having an affinity to Fc region of human IgG
  misc_feature (1)..(3): Xaa can be any naturally occurring amino acid
  MISC_FEATURE (8)..(8): Xaa is lysine, cystein, aspartic acid, glutamic acid, 2-amino suberic acid, or diaminopropionic acid
  misc_feature (15)..(17): Xaa can be any naturally occurring amino acid
XXXCAYHXGELVWCXXX

SEQ ID NO: 101 - protein, 13 aa, Artificial Sequence
  Peptide having an affinity to Fc region of human IgG
  MISC_FEATURE (3)..(3): Xaa is alanine, or threonine
  MISC_FEATURE (4)..(4): Xaa is tyrosine, or tryptophan
  MISC_FEATURE (6)..(6): Xaa is lysine, cystein, aspartic acid, glutamic acid, 2-amino suberic acid, or diaminopropionic acid
  MISC_FEATURE (8)..(8): Xaa is glutamic acid, or aspartic acid
DCXXHXGXLVWCT

SEQ ID NO: 102 - protein, 17 aa, Artificial Sequence
  Peptide having an affinity to Fc region of human IgG
  misc_feature (1)..(3): Xaa can be any naturally occurring amino acid
  MISC_FEATURE (5)..(5): Xaa is alanine, or lysine
  MISC_FEATURE (6)..(6): Xaa is tryptophan, or tyrosine
  MISC_FEATURE (8)..(8): Xaa is arginine, leucine, lysine, aspartic acid, glutamic acid, 2-amino suberic acid, or diaminopropionic acid
  MISC_FEATURE (10)..(10): Xaa is lysine, glutamine, glutamic acid, asparagine, or aspartic acid
  MISC_FEATURE (15)..(15): Xaa is threonine, or lysine
  MISC_FEATURE (16)..(16): Xaa is tyrosine, lysine, or absence
  MISC_FEATURE (17)..(17): Xaa is histidine, lysine, or absence
XXXCXXHXGXLVWCXXX

SEQ ID NO: 103 - protein, 15 aa, Artificial Sequence
  Peptide having an affinity to Fc region of human IgG
  MISC_FEATURE (3)..(3): Xaa is alanine, or lysine
  MISC_FEATURE (4)..(4): Xaa is tryptophan, or tyrosine
  MISC_FEATURE (6)..(6): Xaa is arginine, leucine, lysine, aspartic acid, glutamic acid, 2-amino suberic acid, or diaminopropionic acid
  MISC_FEATURE (8)..(8): Xaa is lysine, glutamine, glutamic acid, asparagine, or aspartic acid
  MISC_FEATURE (13)..(13): Xaa is threonine, or lysine
  MISC_FEATURE (14)..(14): Xaa is tyrosine, lysine, or absence
  MISC_FEATURE (15)..(15): Xaa is histidine, lysine, or absence
DCXXHXGXLVWCXXX

SEQ ID NO: 104 - protein, 13 aa, Artificial Sequence
  Peptide having an affinity to Fc region of human IgG
  MISC_FEATURE (3)..(3): Xaa is alanine, or lysine
  MISC_FEATURE (4)..(4): Xaa is tryptophan, or tyrosine
  MISC_FEATURE (6)..(6): Xaa is arginine, leucine, lysine, cystein, aspartic acid, glutamic acid, 2-amino suberic acid, or diaminopropionic acid
  MISC_FEATURE (8)..(8): Xaa is lysine, glutamine, glutamic acid, asparagine, or aspartic acid
DCXXHXGXLVWCT

SEQ ID NO: 105 - protein, 17 aa, Artificial Sequence
  Peptide having an affinity to Fc region of human IgG
  MISC_FEATURE (5)..(5): Xaa is alanine, or lysine
  MISC_FEATURE (6)..(6): Xaa is Tryptophan, or tyrosine
  MISC_FEATURE (8)..(8): Xaa is arginine, leucine, lysine, aspartic acid, glutamic acid, 2-amino suberic acid, or diaminopropionic acid
  MISC_FEATURE (10)..(10): Xaa is lysine, glutamine, glutamic acid, asparagine, or aspartic acid
  MISC_FEATURE (15)..(15): Xaa is threonine, or lysine
  MISC_FEATURE (16)..(16): Xaa is tyrosine, lysine, or absence
  MISC_FEATURE (17)..(17): Xaa is histidine, lysine, or absence
RGNCXXHXGXLVWCXXX